European Patent Specification EP 3 036 005 B1, published July 1, 2026. Title: COMPOSITIONS AND METHODS FOR TARGETING CONNEXIN HEMICHANNELS. Applicant: Jiang, Jean X. Riquelme, Manuel A. Gu, Sumin. The sequence listing filed with the application follows.

SEQUENCE LISTING (15 sequences)

SEQ ID NO: 1 - DNA, 384 bp, Mus musculus
gaggttcagctggagcagcctggggctgaactggtgaagcctggggcttcagtgaagttgtcctgcaaggcttctggctacaccttcaccagctactatatgtactgggtgaagcagaggcctggacaaggccttgagtggattgggggaattaatcctagcaatggtggtactaacttcaatgagaagttcaagaacaaggccacactgactgtagacaaatcctccagcacagcctacatgcaactcagcagcctgacatctgaggactctgcggtctattactgtacaagagagggtaacccctactatactatgaactactggggtcaaggaacctcagtcaccgtctcctcagccaaaacgacacccccatctgtctat

SEQ ID NO: 2 - protein, 128 aa, Mus musculus
EVQLEQPGAELVKPGASVKLSCKASGYTFTSYYMYWVKQRPGQGLEWIGGINPSNGGTNFNEKFKNKATLTVDKSSSTAYMQLSSLTSEDSAVYYCTREGNPYYTMNYWGQGTSVTVSSAKTTPPSVY

SEQ ID NO: 3 - DNA, 324 bp, Mus musculus
gatattgtgatgacacagactcctgcttccttagctgtatctctggggcagagggccaccatctcatacagggccagcaaaagtgtcagtacatctggctatagttatatgcactggaaccaacagaaaccaggacagccacccagactcctcatctatcttgtatccaacctagaatctggggtccctgccaggttcagtggcagtgggtctgggacagacttcaccctcaacatccatcctgtggaggaggaggatgctgcaacctattactgtcagcacattagggagcttacacgttcggaggggggaccaagctggaaa

SEQ ID NO: 4 - protein, 108 aa, Mus musculus
DIVMTQTPASLAVSLGQRATISYRASKSVSTSGYSYMHWNQQKPGQPPRLLIYLVSNLESGVPARFSGSGSGTDFTLNIHPVEEEDAATYYCQHIRELTRSEGGPSWK

SEQ ID NO: 5 - DNA, 384 bp, Mus musculus; identical to SEQ ID NO: 1

SEQ ID NO: 6 - protein, 128 aa, Mus musculus; identical to SEQ ID NO: 2

SEQ ID NO: 7 - DNA, 375 bp, Mus musculus
gatattgtgatgacccagactccatcctccctgagtgtgtcagcaggagagaaggtcactatgagctgcaagtccagtcagagtctgttaaacagtggaaatcaaaagacctacttggcctggtaccagcagaaaccagggcagcctcctaaactgttgatctacggggcatccactagggaatctggggtccctgatcgcttcacaggcagtggatctggaaccgatttcactcttaccatcagcagtgtgcaggctgaagacctggcagtttattactgtcagaatgatcatagttatccattcacgttcggctcggggacaaagttggaaataaaacgggctgatgctgcaccaactgtatccgcatgcacc

SEQ ID NO: 8 - protein, 122 aa, Mus musculus
DIVMTQTPSSLSVSAGEKVTMSCKSSQSLLNSGNQKTYLAWYQQKPGQPPKLLIYGASTRESGVPDRFTGSGSGTDFTLTISSVQAEDLAVYYCQNDHSYPFTFGSGTKLEIKRADAAPTVS

SEQ ID NO: 9 - DNA, 405 bp, Mus musculus
ctggagcagcctggggctgaactggtgaggcctggggcttcagtaatgctgtcctgcaaggcttctggctacatcttcaccacctactggatgcactggctgaagcagaggcctggacaaggccttgactggattggagagattagtcctagcaacggtcgttctaattacaataagaagttcaagagcaaggccacactgactgtagacaaatcctccagcacagcctacatgcaactcagcagcctgacatctgaggactctgcggtctattactgtgcacgattcgacgagggggacttctggggccaaggcaccactctcatagtctcctcagccaaaacaacagccccatcggtctatccactggcccctgtgtgtggagatacaactggctcctcggtg

SEQ ID NO: 10 - protein, 135 aa, Mus musculus
LEQPGAELVRPGASVMLSCKASGYIFTTYWMHWLKQRPGQGLDWIGEISPSNGRSNYNKKFKSKATLTVDKSSSTAYMQLSSLTSEDSAVYYCARFDEGDFWGQGTTLIVSSAKTTAPSVYPLAPVCGDTTGSSV

SEQ ID NO: 11 - DNA, 324 bp, Mus musculus; identical to SEQ ID NO: 3

SEQ ID NO: 12 - protein, 108 aa, Mus musculus; identical to SEQ ID NO: 4

SEQ ID NO: 13 - protein, 10 aa, Artificial Sequence
  synthetic peptide
FLSRPTEKTI

SEQ ID NO: 14 - protein, 10 aa, Artificial Sequence
  synthetic peptide
KRDPCPHQVD

SEQ ID NO: 15 - protein, 9 aa, Artificial Sequence
  synthetic peptide
LSAVYTCKR